European Patent Application EP 4 534 105 A1, published April 9, 2025. Title: ANTI-CLDN18.2 ANTIBODY, AND ANTIBODY-DRUG CONJUGATE AND USE THEREOF. Applicant: Bio-Thera Solutions, Ltd. The sequence listing filed with the application follows.

SEQUENCE LISTING (88 sequences)

SEQ ID NO: 1 - protein, 5 aa, synthetic construct
SYYIH

SEQ ID NO: 2 - protein, 5 aa, synthetic construct
DYGMH

SEQ ID NO: 3 - protein, 5 aa, synthetic construct
NTYIY

SEQ ID NO: 4 - protein, 5 aa, synthetic construct
DYYMH

SEQ ID NO: 5 - protein, 5 aa, synthetic construct
TSGMS

SEQ ID NO: 6 - protein, 5 aa, synthetic construct
GYWIE

SEQ ID NO: 7 - protein, 17 aa, synthetic construct
WIYPGSGNTKYNEKFKG

SEQ ID NO: 8 - protein, 17 aa, synthetic construct
YISRGRSTTYSTDTVKG

SEQ ID NO: 9 - protein, 17 aa, synthetic construct
RIDPANGNTKYAPKFQG

SEQ ID NO: 10 - protein, 17 aa, synthetic construct
YISSGRSTIYSADTVKG

SEQ ID NO: 11 - protein, 17 aa, synthetic construct
EIYPGSGNTYYNEKFKG

SEQ ID NO: 12 - protein, 17 aa, synthetic construct
LINTYSGVPTYADDFKG

SEQ ID NO: 13 - protein, 17 aa, synthetic construct
EILPGSGSTNYNEKFKG

SEQ ID NO: 14 - protein, 11 aa, synthetic construct
GMDYGNYYLDY

SEQ ID NO: 15 - protein, 10 aa, synthetic construct
GSYYGNAMDY

SEQ ID NO: 16 - protein, 13 aa, synthetic construct
SPAYYINYYAMDY

SEQ ID NO: 17 - protein, 10 aa, synthetic construct
GGYYGNAMDY

SEQ ID NO: 18 - protein, 17 aa, synthetic construct
GGDYYDYDGTGYYAMDY

SEQ ID NO: 19 - protein, 8 aa, synthetic construct
WSRAWFPY

SEQ ID NO: 20 - protein, 12 aa, synthetic construct
APLEGLRSGFAY

SEQ ID NO: 21 - protein, 10 aa, synthetic construct
GSYYGNALDY

SEQ ID NO: 22 - protein, 11 aa, synthetic construct
KASQDVGTAVA

SEQ ID NO: 23 - protein, 11 aa, synthetic construct
HASQNINVWLS

SEQ ID NO: 24 - protein, 10 aa, synthetic construct
SASSSVSYMH

SEQ ID NO: 25 - protein, 11 aa, synthetic construct
KASQNVGTNVA

SEQ ID NO: 26 - protein, 17 aa, synthetic construct
KSSQSLLNSGNQRNYLT

SEQ ID NO: 27 - protein, 12 aa, synthetic construct
SASSSVSSSYLY

SEQ ID NO: 28 - protein, 15 aa, synthetic construct
RASESVDSYGNSFMH

SEQ ID NO: 29 - protein, 11 aa, synthetic construct
RASQSISDYLH

SEQ ID NO: 30 - protein, 7 aa, synthetic construct
WASTRHT

SEQ ID NO: 31 - protein, 7 aa, synthetic construct
KASNLHT

SEQ ID NO: 32 - protein, 7 aa, synthetic construct
DTSKLAS

SEQ ID NO: 33 - protein, 7 aa, synthetic construct
STSYRYS

SEQ ID NO: 34 - protein, 7 aa, synthetic construct
WASTRES

SEQ ID NO: 35 - protein, 7 aa, synthetic construct
STSNLAS

SEQ ID NO: 36 - protein, 7 aa, synthetic construct
RASNLES

SEQ ID NO: 37 - protein, 7 aa, synthetic construct
YASQSIS

SEQ ID NO: 38 - protein, 8 aa, synthetic construct
QQYSSYLT

SEQ ID NO: 39 - protein, 9 aa, synthetic construct
QQGQSYPYT

SEQ ID NO: 40 - protein, 9 aa, synthetic construct
QQWSSNPFT

SEQ ID NO: 41 - protein, 9 aa, synthetic construct
QQYNSYPLT

SEQ ID NO: 42 - protein, 9 aa, synthetic construct
QSAYSYPFT

SEQ ID NO: 43 - protein, 9 aa, synthetic construct
HQWSSYPPT

SEQ ID NO: 44 - protein, 9 aa, synthetic construct
QQSNEDPRT

SEQ ID NO: 45 - protein, 9 aa, synthetic construct
QNGHSFPYT

SEQ ID NO: 46 - protein, 120 aa, synthetic construct
EVQLQESGPELVKPGASVKISCKASGYSFTSYYIHWVKQRPGQGLEWIGWIYPGSGNTKYNEKFKGKATLTADTSSSTAYMQLSSLTSEDSAVYYCARGMDYGNYYLDYWGQGTTLTVSS

SEQ ID NO: 47 - protein, 119 aa, synthetic construct
EVKLQESGGGLVKPGGSLKVSCAASGFTFSDYGMHWVRQAPEKGLEWVAYISRGRSTTYSTDTVKGRFTISRDSAKHTLFLQMTSLRSEDTAMYYCARGSYYGNAMDYWGQGTSVTVSS

SEQ ID NO: 48 - protein, 122 aa, synthetic construct
EVKLQQSVAELVRPGASVKLSCTASGFNIKNTYIYWVKQRPEQGLEWIGRIDPANGNTKYAPKFQGKATITADTSSNTAYLQLSSLTSEDTAIYYCARSPAYYINYYAMDYWGQGTSVTVSS

SEQ ID NO: 49 - protein, 119 aa, synthetic construct
EVQLQESGGGLVKPGGSLKLSCAASGFTFSDYGMHWVRQAPEKGLEWVAYISSGRSTIYSADTVKGRFTISRDNAKNTLFLQMTSLRSEDTAMYYCARGGYYGNAMDYWGQGTSVTVSS

SEQ ID NO: 50 - protein, 126 aa, synthetic construct
EVKLQESGPELVKPGASVKMSCKASGYTFTDYYMHWVKQKPGKGLEWIGEIYPGSGNTYYNEKFKGKATLTADTSSSTAYMQLSSLTSEDSAVYFCAGGGDYYDYDGTGYYAMDYWGQGTSVTVSS

SEQ ID NO: 51 - protein, 110 aa, synthetic construct
EVQLQESGETVKISCKASGYIFTTSGMSWVIQAPGKGLKWMGLINTYSGVPTYADDFKGRFAFSLETSASTAYLQINNLENEDTATYFCAIWSRAWFPYWGQGTLVTVSA

SEQ ID NO: 52 - protein, 121 aa, synthetic construct
EVKLQESGAELMKPGASVKLSCKATGYTFTGYWIEWVKQRPGHGLEWIGEILPGSGSTNYNEKFKGKATFTADTSSNTAYMQLSSLTTEDSAIYYCARAPLEGLRSGFAYWGQGTLVTVSA

SEQ ID NO: 53 - protein, 119 aa, synthetic construct
EVQLLESGGGLVQPGGSLRLSCAASGFTFSDYGMHWVRQAPGKGLEWVAYISRGRSTTYSTDTVKGRFTISRDSSKNTLYLQMNSLRAEDTAVYYCARGSYYGNAMDYWGQGTLVTVSS

SEQ ID NO: 54 - protein, 119 aa, synthetic construct
EVQLLESGGGLVQPGGSLRLSCAASGFTFSDYGMHWVRQAPGKGLEWVAYISRGRSTTYSTDTVKGRFTISRDNSKNTLYLQMNSLRAEDTAVYYCARGSYYGNAMDYWGQGTLVTVSS

SEQ ID NO: 55 - protein, 119 aa, synthetic construct
EVQLLESGGGLVQPGGSLRLSCAASGFTFSDYGMHWVRQAPGKGLEWVAYISRGRSTTYSTDTVKGRFTISRDNSKNTLYLQMNSLRAEDTAVYYCARGSYYGNALDYWGQGTLVTVSS

SEQ ID NO: 56 - protein, 106 aa, synthetic construct
DIVMTQSHKFMSTSVGDRVSITCKASQDVGTAVAWYQQKPGQSPKLLIYWASTRHTGVPDRFTGSGSGTDFTLTISNVQSEDLADYFCQQYSSYLTFGAGTKLELK

SEQ ID NO: 57 - protein, 107 aa, synthetic construct
DIQLTQSPSSLSASLGDTITITCHASQNINVWLSWYQQKPGNIPKLLIYKASNLHTGVPSRFSGSGSGTGFTLTISSLQPEDIATYYCQQGQSYPYTFGGGTKLEIK

SEQ ID NO: 58 - protein, 106 aa, synthetic construct
QIVLTQSPAIMSASPGEKVTMTCSASSSVSYMHWYQQKSGTSPKRWIYDTSKLASGVPARFSGSGSGTSYSLTISSMEAEDAATYYCQQWSSNPFTFGSGTKLEIK

SEQ ID NO: 59 - protein, 107 aa, synthetic construct
DIVMTQSQKFMSTSVGDRVSVTCKASQNVGTNVAWYQLKPGQSPKPLIYSTSYRYSGVPDRFTGSGSGTDFTLTISNVQSEDLAEYFCQQYNSYPLTFGAGTKLELT

SEQ ID NO: 60 - protein, 113 aa, synthetic construct
DIVMTQSPSSLTVTAGERVTMSCKSSQSLLNSGNQRNYLTWYQQKPGQPPKLLIYWASTRESGVPDRFTGSGSGTDFTLTISSVQAEDLAVYFCQSAYSYPFTFGSGTKLEIK

SEQ ID NO: 61 - protein, 108 aa, synthetic construct
QIVLTQSPAIMSASPGEKVTLTCSASSSVSSSYLYWYQQKPGSSPKLWIYSTSNLASGVPARFSGSGSGTSYSLTISSMEAEDAASYFCHQWSSYPPTFGGGTKLEIK

SEQ ID NO: 62 - protein, 111 aa, synthetic construct
DIVLTQSPASLAVSLGQRATISCRASESVDSYGNSFMHWYQQKPGQPPKLLIYRASNLESGIPARFSGSGSRTDFTLTINPVEADDVATYYCQQSNEDPRTFGGGTKLEIK

SEQ ID NO: 63 - protein, 107 aa, synthetic construct
DIVMTQSPATLSVTPGDRVSLSCRASQSISDYLHWYQQKSHESPRLLIKYASQSISGIPSRFSGSGSGSDFTLSINSVEPEDVGVYYCQNGHSFPYTFGGGTKLEIK

SEQ ID NO: 64 - protein, 113 aa, synthetic construct
DIVMTQSPDSLAVSLGERATINCKSSQSLLNSGNQRNYLTWYQQKPGQPPKLLIYWASTRESGVPDRFSGSGSGTDFTLTISSLQAEDVAVYYCQSAYSYPFTFGGGTKLEIK

SEQ ID NO: 65 - protein, 330 aa, synthetic construct [sequence omitted]

SEQ ID NO: 66 - protein, 330 aa, synthetic construct
ASTKGPSVFPLAPSSKSTSGGTAALGCLVKDYFPEPVTVSWNSGALTSGVHTFPAVLQSSGLYSLSSVVTVPSSSLGTQTYICNVNHKPSNTKVDKKVEPKSCDKTHTCPPCPAPELLGGPSVFLFPPKPKDTLMISRTPEVTCVVVDVSHEDPEVKFNWYVDGVEVHNAKTKPREEQYASTYRVVSVLTVLHQDWLNGKEYKCKVSNKALPAPIEKTISKAKGQPREPQVYTLPPSRDELTKNQVSLTCLVKGFYPSDIAVEWESNGQPENNYKTTPPVLDSDGSFFLYSKLTVDKSRWQQGNVFSCSVMHEALHNHYTQKSLSLSPGK

SEQ ID NO: 67 - protein, 330 aa, synthetic construct
ASTKGPSVFPLAPSSKSTSGGTAALGCLVKDYFPEPVTVSWNSGALTSGVHTFPAVLQSSGLYSLSSVVTVPSSSLGTQTYICNVNHKPSNTKVDKKVEPKSCDKTHTCPPCPAPEAAGGPSVFLFPPKPKDTLMISRTPEVTCVVVDVSHEDPEVKFNWYVDGVEVHNAKTKPREEQYNSTYRVVSVLTVLHQDWLNGKEYKCKVSNKALGAPIEKTISKAKGQPREPQVYTLPPSRDELTKNQVSLTCLVKGFYPSDIAVEWESNGQPENNYKTTPPVLDSDGSFFLYSKLTVDKSRWQQGNVFSCSVMHEALHNHYTQKSLSLSPGK

SEQ ID NO: 68 - protein, 107 aa, synthetic construct [sequence omitted]

SEQ ID NO: 69 - protein, 449 aa, synthetic construct
EVQLLESGGGLVQPGGSLRLSCAASGFTFSDYGMHWVRQAPGKGLEWVAYISRGRSTTYSTDTVKGRFTISRDNSKNTLYLQMNSLRAEDTAVYYCARGSYYGNALDYWGQGTLVTVSSASTKGPSVFPLAPSSKSTSGGTAALGCLVKDYFPEPVTVSWNSGALTSGVHTFPAVLQSSGLYSLSSVVTVPSSSLGTQTYICNVNHKPSNTKVDKKVEPKSCDKTHTCPPCPAPELLGGPSVFLFPPKPKDTLMISRTPEVTCVVVDVSHEDPEVKFNWYVDGVEVHNAKTKPREEQYNSTYRVVSVLTVLHQDWLNGKEYKCKVSNKALPAPIEKTISKAKGQPREPQVYTLPPSRDELTKNQVSLTCLVKGFYPSDIAVEWESNGQPENNYKTTPPVLDSDGSFFLYSKLTVDKSRWQQGNVFSCSVMHEALHNHYTQKSLSLSPGK

SEQ ID NO: 70 - protein, 449 aa, synthetic construct
EVQLLESGGGLVQPGGSLRLSCAASGFTFSDYGMHWVRQAPGKGLEWVAYISRGRSTTYSTDTVKGRFTISRDNSKNTLYLQMNSLRAEDTAVYYCARGSYYGNALDYWGQGTLVTVSSASTKGPSVFPLAPSSKSTSGGTAALGCLVKDYFPEPVTVSWNSGALTSGVHTFPAVLQSSGLYSLSSVVTVPSSSLGTQTYICNVNHKPSNTKVDKKVEPKSCDKTHTCPPCPAPELLGGPSVFLFPPKPKDTLMISRTPEVTCVVVDVSHEDPEVKFNWYVDGVEVHNAKTKPREEQYASTYRVVSVLTVLHQDWLNGKEYKCKVSNKALPAPIEKTISKAKGQPREPQVYTLPPSRDELTKNQVSLTCLVKGFYPSDIAVEWESNGQPENNYKTTPPVLDSDGSFFLYSKLTVDKSRWQQGNVFSCSVMHEALHNHYTQKSLSLSPGK

SEQ ID NO: 71 - protein, 449 aa, synthetic construct
EVQLLESGGGLVQPGGSLRLSCAASGFTFSDYGMHWVRQAPGKGLEWVAYISRGRSTTYSTDTVKGRFTISRDNSKNTLYLQMNSLRAEDTAVYYCARGSYYGNALDYWGQGTLVTVSSASTKGPSVFPLAPSSKSTSGGTAALGCLVKDYFPEPVTVSWNSGALTSGVHTFPAVLQSSGLYSLSSVVTVPSSSLGTQTYICNVNHKPSNTKVDKKVEPKSCDKTHTCPPCPAPEAAGGPSVFLFPPKPKDTLMISRTPEVTCVVVDVSHEDPEVKFNWYVDGVEVHNAKTKPREEQYNSTYRVVSVLTVLHQDWLNGKEYKCKVSNKALGAPIEKTISKAKGQPREPQVYTLPPSRDELTKNQVSLTCLVKGFYPSDIAVEWESNGQPENNYKTTPPVLDSDGSFFLYSKLTVDKSRWQQGNVFSCSVMHEALHNHYTQKSLSLSPGK

SEQ ID NO: 72 - protein, 220 aa, synthetic construct
DIVMTQSPDSLAVSLGERATINCKSSQSLLNSGNQRNYLTWYQQKPGQPPKLLIYWASTRESGVPDRFSGSGSGTDFTLTISSLQAEDVAVYYCQSAYSYPFTFGGGTKLEIKRTVAAPSVFIFPPSDEQLKSGTASVVCLLNNFYPREAKVQWKVDNALQSGNSQESVTEQDSKDSTYSLSSTLTLSKADYEKHKVYACEVTHQGLSSPVTKSFNRGEC

SEQ ID NO: 73 - DNA, 660 bp, synthetic construct
  source 1..660: mol_type = other DNA
gacatcgtgatgacccagtctccagattctctggcagtgtctctgggagaaagagctacaatcaactgcaagtcctctcagtctctgctgaactccggcaaccagagaaactacctgacttggtaccagcagaaaccaggacagcctcctaagctgctgatctattgggcttctaccagggaatccggagtgccagatagattttccggatctggatccggcaccgattttacactgacaatctcttctctgcaggcagaagacgtggctgtgtattattgccagtccgcctactcctacccttttacctttggcggaggaacaaagctggagatcaagcgtacggtggctgcaccatctgtcttcatcttcccgccatctgatgagcagttgaaatctggaactgcctctgttgtgtgcctgctgaataacttctatcccagagaggccaaagtacagtggaaggtggataacgccctccaatcgggtaactcccaggagagtgtcacagagcaggacagcaaggacagcacctacagcctcagcagcaccctgacgctgagcaaagcagactacgagaaacacaaagtctacgcctgcgaagtcacccatcagggcctgagctcgcccgtcacaaagagcttcaacaggggagagtgt

SEQ ID NO: 74 - DNA, 1347 bp, synthetic construct
  source 1..1347: mol_type = other DNA
gaagtgcaacttcttgaatctggaggaggacttgtgcaacctggaggatctcttagactttcttgcgcagcatctggatttacattcagcgactatggaatgcattgggtgagacaagcacctggaaagggtctagaatgggtggcatatatctctagaggaagatctacaacatattctacagatacagtgaaaggaagatttacaatctctagagataactctaagaataccctttatcttcaaatgaactctcttagagcagaagatacagcagtgtattattgcgcaagaggatcttattatggaaacgcacttgattattgggggcagggaacacttgtgacagtgtcttctgcatctacaaagggtcctagcgtgtttcctcttgcaccttcttctaaatctacatctggaggaacagcagcacttggatgccttgtgaaagattatttccccgaaccggtgacggtgtcgtggaactcaggcgccctgaccagcggcgtgcacaccttcccggctgtcctacagtcctcaggactctactccctcagcagcgtggtgaccgtgccctccagcagcttgggcacccagacctacatctgcaacgtgaatcacaagcccagcaacaccaaggtggacaagaaagttgagcccaaatcttgtgacaaaactcacacatgcccaccgtgcccagcacctgaactcctggggggaccgtcagtcttcctcttccccccaaaacccaaggacaccctcatgatctcccggacccctgaggtcacatgcgtggtggtggacgtgagccacgaagaccctgaggtcaagttcaactggtacgtggacggcgtggaggtgcataatgccaagacaaagccgcgggaggagcagtacaacagcacgtaccgtgtggtcagcgtcctcaccgtcctgcaccaggactggctgaatggcaaggagtacaagtgcaaggtctccaacaaagccctcccagcccccatcgagaaaaccatctccaaagccaaagggcagccccgagaaccacaggtgtacaccctgcccccatcccgggatgagctgaccaagaaccaggtcagcctgacctgcctggtcaaaggcttctatcccagcgacatcgccgtggagtgggagagcaatgggcagccggagaacaactacaagaccacgcctcccgtgctggactccgacggctccttcttcctctacagcaagctcaccgtggacaagagcaggtggcagcaggggaacgtcttctcatgctccgtgatgcatgaggctctgcacaaccactacacgcagaagagcctctccctgtctccgggtaaa

SEQ ID NO: 75 - DNA, 1347 bp, synthetic construct
  source 1..1347: mol_type = other DNA
gaagtgcaacttcttgaatctggaggaggacttgtgcaacctggaggatctcttagactttcttgcgcagcatctggatttacattcagcgactatggaatgcattgggtgagacaagcacctggaaagggtctagaatgggtggcatatatctctagaggaagatctacaacatattctacagatacagtgaaaggaagatttacaatctctagagataactctaagaataccctttatcttcaaatgaactctcttagagcagaagatacagcagtgtattattgcgcaagaggatcttattatggaaacgcacttgattattgggggcagggaacacttgtgacagtgtcttctgcatctacaaagggtcctagcgtgtttcctcttgcaccttcttctaaatctacatctggaggaacagcagcacttggatgccttgtgaaagattatttccccgaaccggtgacggtgtcgtggaactcaggcgccctgaccagcggcgtgcacaccttcccggctgtcctacagtcctcaggactctactccctcagcagcgtggtgaccgtgccctccagcagcttgggcacccagacctacatctgcaacgtgaatcacaagcccagcaacaccaaggtggacaagaaagttgagcccaaatcttgtgacaaaactcacacatgcccaccgtgcccagcacctgaactcctggggggaccgtcagtcttcctcttccccccaaaacccaaggacaccctcatgatctcccggacccctgaggtcacatgcgtggtggtggacgtgagccacgaagaccctgaggtcaagttcaactggtacgtggacggcgtggaggtgcataatgccaagacaaagccgcgggaggagcagtacgccagcacgtaccgtgtggtcagcgtcctcaccgtcctgcaccaggactggctgaatggcaaggagtacaagtgcaaggtctccaacaaagccctcccagcccccatcgagaaaaccatctccaaagccaaagggcagccccgagaaccacaggtgtacaccctgcccccatcccgggatgagctgaccaagaaccaggtcagcctgacctgcctggtcaaaggcttctatcccagcgacatcgccgtggagtgggagagcaatgggcagccggagaacaactacaagaccacgcctcccgtgctggactccgacggctccttcttcctctacagcaagctcaccgtggacaagagcaggtggcagcaggggaacgtcttctcatgctccgtgatgcatgaggctctgcacaaccactacacgcagaagagcctctccctgtctccgggtaaa

SEQ ID NO: 76 - DNA, 1347 bp, synthetic construct
  source 1..1347: mol_type = other DNA
gaagtgcaacttcttgaatctggaggaggacttgtgcaacctggaggatctcttagactttcttgcgcagcatctggatttacattcagcgactatggaatgcattgggtgagacaagcacctggaaagggtctagaatgggtggcatatatctctagaggaagatctacaacatattctacagatacagtgaaaggaagatttacaatctctagagataactctaagaataccctttatcttcaaatgaactctcttagagcagaagatacagcagtgtattattgcgcaagaggatcttattatggaaacgcacttgattattgggggcagggaacacttgtgacagtgtcttctgcctctacaaaggggcctagtgtatttccactggccccttcttctaaatccaccagtggtggtacggcagcactcggttgcctggtgaaggattacttcccggaaccggtcaccgtaagttggaactcaggcgctcttaccagcggagttcacacctttccagccgtgctgcagagctccgggctgtattctctgtcctctgtggtgaccgttcctagttcctccctgggaacacagacctacatatgcaacgtgaatcataagccaagcaacactaaggtcgacaaaaaggtggagcccaagagctgtgacaagacccacacctgtccgccatgtccagcccctgaagctgcaggaggtccatcagtgttcctgttccctccgaagccaaaggacaccctgatgatctcacgaactcccgaagtgacttgcgtcgtggtggacgtgagtcacgaagaccccgaagtcaagttcaattggtatgtcgatggcgttgaggttcacaatgcaaagaccaagccaagagaggagcagtacaactcaacataccgggttgtgtctgtgctgaccgtgctgcatcaggattggttgaacgggaaagagtataaatgcaaagttagcaacaaggcactcggtgctccaatagagaagaccataagcaaggctaaggggcagccacgcgaacctcaggtttacaccttgcctccatctagggatgaactgactaaaaaccaagtcagcctgacatgcctcgtgaagggattctatccttctgacattgcagtcgagtgggagtccaacggccagccagaaaacaactacaaaacaactcctcctgtgctcgacagcgacggatctttctttctctattccaagttgactgtggacaaaagccgctggcagcaggggaacgtcttctcttgctccgtgatgcacgaggccttgcataaccattacacccagaaatctctctcactgtctccaggcaaa

SEQ ID NO: 77 - skipped

SEQ ID NO: 78 - protein, 22 aa, synthetic construct
MDMRVLAQLLGLLLLCFPGARC

SEQ ID NO: 79 - DNA, 66 bp, synthetic construct
  source 1..66: mol_type = other DNA
atggacatgagggtgctggcccagctgctgggactgctgctgctgtgcttcccaggcgccagatgc

SEQ ID NO: 80 - protein, 19 aa, synthetic construct
MGWSLILLFLVAVATRVLS

SEQ ID NO: 81 - DNA, 57 bp, synthetic construct
  source 1..57: mol_type = other DNA
atgggttggtctcttatccttctattcctggttgcagtggcaacaagagtgctttct

SEQ ID NO: 82 - DNA, 57 bp, synthetic construct
  source 1..57: mol_type = other DNA
atgggttggtctctgattctcctgtttctggtggcagtggctacaagagtcctgtca

SEQ ID NO: 83 - protein, 451 aa, synthetic construct
QVQLQQSGSELKKPGASVKVSCKASGYTFTNYGMNWVKQAPGQGLKWMGWINTYTGEPTYTDDFKGRFAFSLDTSVSTAYLQISSLKADDTAVYFCARGGFGSSYWYFDVWGQGTLVTVSSASTKGPSVFPLAPSSKSTSGGTAALGCLVKDYFPEPVTVSWNSGALTSGVHTFPAVLQSSGLYSLSSVVTVPSSSLGTQTYICNVNHKPSNTKVDKKVEPKSCDKTHTCPPCPAPELLGGPSVFLFPPKPKDTLMISRTPEVTCVVVDVSHEDPEVKFNWYVDGVEVHNAKTKPREEQYNSTYRVVSVLTVLHQDWLNGKEYKCKVSNKALPAPIEKTISKAKGQPREPQVYTLPPSRDELTKNQVSLTCLVKGFYPSDIAVEWESNGQPENNYKTTPPVLDSDGSFFLYSKLTVDKSRWQQGNVFSCSVMHEALHNHYTQKSLSLSPGK

SEQ ID NO: 84 - protein, 214 aa, synthetic construct
DIQLTQSPSSLSASVGDRVSITCKASQDVSIAVAWYQQKPGKAPKLLIYSASYRYTGVPDRFSGSGSGTDFTLTISSLQPEDFAVYYCQQHYITPLTFGAGTKVEIKRTVAAPSVFIFPPSDEQLKSGTASVVCLLNNFYPREAKVQWKVDNALQSGNSQESVTEQDSKDSTYSLSSTLTLSKADYEKHKVYACEVTHQGLSSPVTKSFNRGEC

SEQ ID NO: 85 - protein, 261 aa, synthetic construct
MAVTACQGLGFVVSLIGIAGIIAATCMDQWSTQDLYNNPVTAVFNYQGLWRSCVRESSGFTECRGYFTLLGLPAMLQAVRALMIVGIVLGAIGLLVSIFALKCIRIGSMEDSAKANMTLTSGIMFIVSGLCAIAGVSVFANMLVTNFWMSTANMYTGMGGMVQTVQTRYTFGAALFVGWVAGGLTLIGGVMMCIACRGLAPEETNYKAVSYHASGHSVAYKPGGFKASTGFGSNTKNKKIYDGGARTEDEVQSYPSKHDYV

SEQ ID NO: 86 - DNA, 783 bp, synthetic construct
  source 1..783: mol_type = other DNA
atggccgtgactgcctgtcagggcttggggttcgtggtttcactgattgggattgcgggcatcattgctgccacctgcatggaccagtggagcacccaagacttgtacaacaaccccgtaacagctgttttcaactaccaggggctgtggcgctcctgtgtccgagagagctctggcttcaccgagtgccggggctacttcaccctgctggggctgccagccatgctgcaggcagtgcgagccctgatgatcgtaggcatcgtcctgggtgccattggcctcctggtatccatctttgccctgaaatgcatccgcattggcagcatggaggactctgccaaagccaacatgacactgacctccgggatcatgttcattgtctcaggtctttgtgcaattgctggagtgtctgtgtttgccaacatgctggtgactaacttctggatgtccacagctaacatgtacaccggcatgggtgggatggtgcagactgttcagaccaggtacacatttggtgcggctctgttcgtgggctgggtcgctggaggcctcacactaattgggggtgtgatgatgtgcatcgcctgccggggcctggcaccagaagaaaccaactacaaagccgtttcttatcatgcctcaggccacagtgttgcctacaagcctggaggcttcaaggccagcactggctttgggtccaacaccaaaaacaagaagatatacgatggaggtgcccgcacagaggacgaggtacaatcttatccttccaagcacgactatgtg

SEQ ID NO: 87 - protein, 261 aa, synthetic construct
MSTTTCQVVAFLLSILGLAGCIAATGMDMWSTQDLYDNPVTSVFQYEGLWRSCVRQSSGFTECRPYFTILGLPAMLQAVRALMIVGIVLGAIGLLVSIFALKCIRIGSMEDSAKANMTLTSGIMFIVSGLCAIAGVSVFANMLVTNFWMSTANMYTGMGGMVQTVQTRYTFGAALFVGWVAGGLTLIGGVMMCIACRGLAPEETNYKAVSYHASGHSVAYKPGGFKASTGFGSNTKNKKIYDGGARTEDEVQSYPSKHDYV

SEQ ID NO: 88 - DNA, 783 bp, synthetic construct
  source 1..783: mol_type = other DNA
atgtccaccaccacatgccaagtggtggcgttcctcctgtccatcctggggctggccggctgcatcgcggccaccgggatggacatgtggagcacccaggacctgtacgacaaccccgtcacctccgtgttccagtacgaagggctctggaggagctgcgtgaggcagagttcaggcttcaccgaatgcaggccctatttcaccatcctgggacttccagccatgctgcaggcagtgcgagccctgatgatcgtaggcatcgtcctgggtgccattggcctcctggtatccatctttgccctgaaatgcatccgcattggcagcatggaggactctgccaaagccaacatgacactgacctccgggatcatgttcattgtctcaggtctttgtgcaattgctggagtgtctgtgtttgccaacatgctggtgactaacttctggatgtccacagctaacatgtacaccggcatgggtgggatggtgcagactgttcagaccaggtacacatttggtgcggctctgttcgtgggctgggtcgctggaggcctcacactaattgggggtgtgatgatgtgcatcgcctgccggggcctggcaccagaagaaaccaactacaaagccgtttcttatcatgcctcaggccacagtgttgcctacaagcctggaggcttcaaggccagcactggctttgggtccaacaccaaaaacaagaagatatacgatggaggtgcccgcacagaggacgaggtacaatcttatccttccaagcacgactatgtg